European Patent Specification EP 4 138 883 B1, published September 10, 2025. Title: A chimeric endolysin polypeptide. Applicant: Micreos Human Health B.V. The sequence listing filed with the application follows.

SEQUENCE LISTING (83 sequences)

SEQ ID NO: 1 - protein, 145 aa, Artificial Sequence
  CHAP-Tw
MKTLKQAESYIKSKVNTGTDFDGLYGYQCMDLAVDYIYHVTDGKIRMWGNAKDAINNSFGGTATVYKNYPAFRPKYGDVVVWTTGNFATYGHIAIVTNPDPYGDLQYVTVLEQNWNGNGIYKTELATIRTHDYTGITHFIRPNFA

SEQ ID NO: 2 - protein, 140 aa, Artificial Sequence
  M23-LST
AATHEHSAQWLNNYKKGYGYGPYPLGINGGMHYGVDFFMNIGTPVKAISSGKIVEAGWSNYGGGNQIGLIENDGVHRQWYMHLSKYNVKVGDYVKAGQIIGWSGSTGYSTAPHLHFQRMVNSFSNSTAQDPMPFLKSAGY

SEQ ID NO: 3 - protein, 94 aa, Artificial Sequence
  SH3b-2638
WKQNKDGIWYKAEHASFTVTAPEGIITRYKGPWTGHPQAGVLQKGQTIKYDEVQKFDGHVWVSWETFEGETVYMPVRTWDAKTGKVGKLWGEIK

SEQ ID NO: 4 - protein, 273 aa, Artificial Sequence
  CHAPTw_SH3b2638
MKTLKQAESYIKSKVNTGTDFDGLYGYQCMDLAVDYIYHVTDGKIRMWGNAKDAINNSFGGTATVYKNYPAFRPKYGDVVVWTTGNFATYGHIAIVTNPDPYGDLQYVTVLEQNWNGNGIYKTELATIRTHDYTGITHFIRPNFAGGKLEVSKAATIKQSDVKQEVKKQEAKQIVKATDWKQNKDGIWYKAEHASFTVTAPEGIITRYKGPWTGHPQAGVLQKGQTIKYDEVQKFDGHVWVSWETFEGETVYMPVRTWDAKTGKVGKLWGEIK

SEQ ID NO: 5 - protein, 439 aa, Artificial Sequence
  CHAPTw_M23LST_SH3b2638
MKTLKQAESYIKSKVNTGTDFDGLYGYQCMDLAVDYIYHVTDGKIRMWGNAKDAINNSFGGTATVYKNYPAFRPKYGDVVVWTTGNFATYGHIAIVTNPDPYGDLQYVTVLEQNWNGNGIYKTELATIRTHDYTGITHFIRPNFATESSVKKKDTKKKPKPSNRDGINKDKAATHEHSAQWLNNYKKGYGYGPYPLGINGGMHYGVDFFMNIGTPVKAISSGKIVEAGWSNYGGGNQIGLIENDGVHRQWYMHLSKYNVKVGDYVKAGQIIGWSGSTGYSTAPHLHFQRMVNSFSNSTAQDPMPFLKSAGYGGKLEVSKAATIKQSDVKQEVKKQEAKQIVKATDWKQNKDGIWYKAEHASFTVTAPEGIITRYKGPWTGHPQAGVLQKGQTIKYDEVQKFDGHVWVSWETFEGETVYMPVRTWDAKTGKVGKLWGEIK

SEQ ID NO: 6 - protein, 428 aa, Artificial Sequence
  M23LST_CHAPTw_SH3b2638
MAATHEHSAQWLNNYKKGYGYGPYPLGINGGMHYGVDFFMNIGTPVKAISSGKIVEAGWSNYGGGNQIGLIENDGVHRQWYMHLSKYNVKVGDYVKAGQIIGWSGSTGYSTAPHLHFQRMVNSFSNSTAQDPMPFLKSAGYGKAGGTVTPTPNTGMKTLKQAESYIKSKVNTGTDFDGLYGYQCMDLAVDYIYHVTDGKIRMWGNAKDAINNSFGGTATVYKNYPAFRPKYGDVVVWTTGNFATYGHIAIVTNPDPYGDLQYVTVLEQNWNGNGIYKTELATIRTHDYTGITHFIRPNFAGGKLEVSKAATIKQSDVKQEVKKQEAKQIVKATDWKQNKDGIWYKAEHASFTVTAPEGIITRYKGPWTGHPQAGVLQKGQTIKYDEVQKFDGHVWVSWETFEGETVYMPVRTWDAKTGKVGKLWGEIK

SEQ ID NO: 7 - protein, 137 aa, Artificial Sequence
  CHAPK
SLKKYNGKLPKHDPSFVQPGNRHYKYQCTWYAYNRRGQLGIPVPLWGDAADWIGGAKGAGYGVGRTPKQGACVIWQRGVQGGSPQYGHVAFVEKVLDGGKKIFISEHNYATPNGYGTRTIDMSSAIGKNAQFIYDKK

SEQ ID NO: 8 - protein, 94 aa, Artificial Sequence; identical to SEQ ID NO: 3
  M23-2638

SEQ ID NO: 9 - protein, 92 aa, Artificial Sequence
  SH3b-LST
WKTNKYGTLYKSESASFTPNTDIITRTTGPFRSMPQSGVLKAGQTIHYDEVMKQDGHVWVGYTGNSGQRIYLPVRTWNKSTNTLGVLWGTIK

SEQ ID NO: 10 - protein, 92 aa, Artificial Sequence
  SH3b-ALE1
YKTNKYGTLYKSESASFTANTDIITRLTGPFRSMPQSGVLRKGLTIKYDEVMKQDGHVWVGYNTNSGKRVYLPVRTWNESTGELGPLWGTIK

SEQ ID NO: 11 - protein, 143 aa, Artificial Sequence
  CHAP-SEP
MKTKKQALKWILNTIGQGIDWDKMYGFQCMDLVVAYLYYVTDGKIAMWGNAIDAPKNNFKGTAKVIKNYPAFRPEEGDIVVWSYGNFSTYGHIAVVIDGDPYGDLQYITVAEQNWNGLGLYKQEVTTKRIHNYDGVSHFIRPK

SEQ ID NO: 12 - protein, 165 aa, Artificial Sequence
  CHAP-GH15
MAKTQAEINKRLDAYAKGTVDSPYRIKKATSYDPSFGVMEAGAIDADGYYHAQCQDLITDYVLWLTDNKVRTWGNAKDQIKQSYGTGFKIHENKPSTVPKKGWIAVFTSGSYQQWGHIGIVYDGGNTSTFTILEQNWNGYANKKPTKRVDNYYGLTHFIEIPVKA

SEQ ID NO: 13 - protein, 117 aa, Artificial Sequence
  TCHAP-K
GNPNTGQWARECTWYCYNRRYELGLKAVAYGDAADWIAGARGAGISTGKEPKRGAVAVWARGVPGGSAQYGHVAFVEKVTDDGIYVSDYNYASPKTYGERLYKKGSPEYRNAQYIYD

SEQ ID NO: 14 - protein, 141 aa, Artificial Sequence
  M23-ALE1
AAQSNHSASWLNNYKKGYGYGPYPLGINGGNHYGVDFFMNVGTPVRAISDGKIVEAGWTNYGGGNEIGLVENDGVHRQWYMHLSKFNVKVGDRVKAGQIIGWSGSTGYSTAPHLHFQRMTNSFSNNTAQDPMPFLKSAGYG

SEQ ID NO: 15 - protein, 135 aa, Artificial Sequence
  TCHAPTw
GKELPTPRNKTDTSWTAPGNPNTGQWARECTWYCYNRRYELGLKAVAYGDAADWIAGARGAGISTGKEPKRGAVAVWARGVPGGSAQYGHVAFVEKVTDDGIYVSDYNYASPKTYGERLYKKGSPEYRNAQYIYD

SEQ ID NO: 16 - protein, 26 aa, Artificial Sequence
  CHAP-Tw C-terminal linker
TESSVKKKDTKKKPKPSNRDGINKDK

SEQ ID NO: 17 - protein, 14 aa, Artificial Sequence
  M23-LST C-terminal linker
GKAGGTVTPTPNTG

SEQ ID NO: 18 - protein, 34 aa, Artificial Sequence
  SH3b-2683 N-terminal linker
GGKLEVSKAATIKQSDVKQEVKKQEAKQIVKATD

SEQ ID NO: 19 - protein, 32 aa, Artificial Sequence
  CHAP-SEP C-terminal linker
FKKTVKKEDNTLTKEKNNKKTKGKKLKVSTQR

SEQ ID NO: 20 - protein, 23 aa, Artificial Sequence
  CHAP-GH15 C-terminal linker
GTTVKKETAKKSASKTPAPKKKA

SEQ ID NO: 21 - protein, 18 aa, Artificial Sequence
  TCHAP-Tw N-terminal linker
GKELPTPRNKTDTSWTAP

SEQ ID NO: 22 - protein, 11 aa, Artificial Sequence
  M23-ALE1 C-terminal linker
SNSTSSSNNNG

SEQ ID NO: 23 - protein, 12 aa, Artificial Sequence
  SH3b-ALE-1 N-terminal Linker
GSNSTSSSNNNG

SEQ ID NO: 24 - protein, 422 aa, Artificial Sequence
  CHAPGH15_M23Ale1_SH3b2638
AKTQAEINKRLDAYAKGTVDSPYRIKKATSYDPSFGVMEAGAIDADGYYHAQCQDLITDYVLWLTDNKVRTWGNAKDQIKQSYGTGFKIHENKPSTVPKKGWIAVFTSGSYQQWGHIGIVYDGGNTSTFTILEQNWNGYANKKPTKRVDNYYGLTHFIEIPVKAGSNSTSSSNNNGAAQSNHSASWLNNYKKGYGYGPYPLGINGGNHYGVDFFMNVGTPVRAISDGKIVEAGWTNYGGGNEIGLVENDGVHRQWYMHLSKFNVKVGDRVKAGQIIGWSGSTGYSTAPHLHFQRMTNSFSNNTAQDPMPFLKSAGYGSNSTSSSNNNGWKQNKDGIWYKAEHASFTVTAPEGIITRYKGPWTGHPQAGVLQKGQTIKYDEVQKFDGHVWVSWETFEGETVYMPVRTWDAKTGKVGKLWGEIK

SEQ ID NO: 25 - protein, 420 aa, Artificial Sequence
  CHAPGH15_M23Ale1_SH3bAle1v
AKTQAEINKRLDAYAKGTVDSPYRIKKATSYDPSFGVMEAGAIDADGYYHAQCQDLITDYVLWLTDNKVRTWGNAKDQIKQSYGTGFKIHENKPSTVPKKGWIAVFTSGSYQQWGHIGIVYDGGNTSTFTILEQNWNGYANKKPTKRVDNYYGLTHFIEIPVKAGSNSTSSSNNNGAAQSNHSASWLNNYKKGYGYGPYPLGINGGNHYGVDFFMNVGTPVRAISDGKIVEAGWTNYGGGNEIGLVENDGVHRQWYMHLSKFNVKVGDRVKAGQIIGWSGSTGYSTAPHLHFQRMTNSFSNNTAQDPMPFLKSAGYGSNSTSSSNNNGYKTNKYGTLYKSESASFTANTDIITRLTGPFRSMPQSGVLRKGLTIKYDEVMKQDGHVWVGYNTNSGKRVYLPVRTWNESTGELGPLWGTIK

SEQ ID NO: 26 - protein, 420 aa, Artificial Sequence
  CHAPGH15_M23Ale1_SH3bLST
AKTQAEINKRLDAYAKGTVDSPYRIKKATSYDPSFGVMEAGAIDADGYYHAQCQDLITDYVLWLTDNKVRTWGNAKDQIKQSYGTGFKIHENKPSTVPKKGWIAVFTSGSYQQWGHIGIVYDGGNTSTFTILEQNWNGYANKKPTKRVDNYYGLTHFIEIPVKAGSNSTSSSNNNGAAQSNHSASWLNNYKKGYGYGPYPLGINGGNHYGVDFFMNVGTPVRAISDGKIVEAGWTNYGGGNEIGLVENDGVHRQWYMHLSKFNVKVGDRVKAGQIIGWSGSTGYSTAPHLHFQRMTNSFSNNTAQDPMPFLKSAGYGSNSTSSSNNNGWKTNKYGTLYKSESASFTPNTDIITRTTGPFRSMPQSGVLKAGQTIHYDEVMKQDGHVWVGYTGNSGQRIYLPVRTWNKSTNTLGVLWGTIK

SEQ ID NO: 27 - protein, 422 aa, Artificial Sequence
  CHAPGH15_M23LST_SH3b2638
AKTQAEINKRLDAYAKGTVDSPYRIKKATSYDPSFGVMEAGAIDADGYYHAQCQDLITDYVLWLTDNKVRTWGNAKDQIKQSYGTGFKIHENKPSTVPKKGWIAVFTSGSYQQWGHIGIVYDGGNTSTFTILEQNWNGYANKKPTKRVDNYYGLTHFIEIPVKAGSNSTSSSNNNGAATHEHSAQWLNNYKKGYGYGPYPLGINGGMHYGVDFFMNIGTPVKAISSGKIVEAGWSNYGGGNQIGLIENDGVHRQWYMHLSKYNVKVGDYVKAGQIIGWSGSTGYSTAPHLHFQRMVNSFSNSTAQDPMPFLKSAGYGSNSTSSSNNNGWKQNKDGIWYKAEHASFTVTAPEGIITRYKGPWTGHPQAGVLQKGQTIKYDEVQKFDGHVWVSWETFEGETVYMPVRTWDAKTGKVGKLWGEIK

SEQ ID NO: 28 - protein, 420 aa, Artificial Sequence
  CHAPGH15_M23LST_SH3bAle1
AKTQAEINKRLDAYAKGTVDSPYRIKKATSYDPSFGVMEAGAIDADGYYHAQCQDLITDYVLWLTDNKVRTWGNAKDQIKQSYGTGFKIHENKPSTVPKKGWIAVFTSGSYQQWGHIGIVYDGGNTSTFTILEQNWNGYANKKPTKRVDNYYGLTHFIEIPVKAGSNSTSSSNNNGAATHEHSAQWLNNYKKGYGYGPYPLGINGGMHYGVDFFMNIGTPVKAISSGKIVEAGWSNYGGGNQIGLIENDGVHRQWYMHLSKYNVKVGDYVKAGQIIGWSGSTGYSTAPHLHFQRMVNSFSNSTAQDPMPFLKSAGYGSNSTSSSNNNGYKTNKYGTLYKSESASFTANTDIITRLTGPFRSMPQSGVLRKGLTIKYDEVMKQDGHVWVGYNTNSGKRVYLPVRTWNESTGELGPLWGTIK

SEQ ID NO: 29 - protein, 420 aa, Artificial Sequence
  CHAPGH15_M23LST_SH3bLST
AKTQAEINKRLDAYAKGTVDSPYRIKKATSYDPSFGVMEAGAIDADGYYHAQCQDLITDYVLWLTDNKVRTWGNAKDQIKQSYGTGFKIHENKPSTVPKKGWIAVFTSGSYQQWGHIGIVYDGGNTSTFTILEQNWNGYANKKPTKRVDNYYGLTHFIEIPVKAGSNSTSSSNNNGAATHEHSAQWLNNYKKGYGYGPYPLGINGGMHYGVDFFMNIGTPVKAISSGKIVEAGWSNYGGGNQIGLIENDGVHRQWYMHLSKYNVKVGDYVKAGQIIGWSGSTGYSTAPHLHFQRMVNSFSNSTAQDPMPFLKSAGYGSNSTSSSNNNGWKTNKYGTLYKSESASFTPNTDIITRTTGPFRSMPQSGVLKAGQTIHYDEVMKQDGHVWVGYTGNSGQRIYLPVRTWNKSTNTLGVLWGTIK

SEQ ID NO: 30 - protein, 404 aa, Artificial Sequence
  CHAPSEP_M23Ale1_SH3b2638
MKTKKQALKWILNTIGQGIDWDKMYGFQCMDLVVAYLYYVTDGKIAMWGNAIDAPKNNFKGTAKVIKNYPAFRPEEGDIVVWSYGNFSTYGHIAVVIDGDPYGDLQYITVAEQNWNGLGLYKQEVTTKRIHNYDGVSHFIRPKFKKTSNSTSSSNNNGAAQSNHSASWLNNYKKGYGYGPYPLGINGGNHYGVDFFMNVGTPVRAISDGKIVEAGWTNYGGGNEIGLVENDGVHRQWYMHLSKFNVKVGDRVKAGQIIGWSGSTGYSTAPHLHFQRMTNSFSNNTAQDPMPFLKSAGYGSNSTSSSNNNGWKQNKDGIWYKAEHASFTVTAPEGIITRYKGPWTGHPQAGVLQKGQTIKYDEVQKFDGHVWVSWETFEGETVYMPVRTWDAKTGKVGKLWGEIK

SEQ ID NO: 31 - protein, 402 aa, Artificial Sequence
  CHAPSEP_M23Ale1_SH3bAle1
MKTKKQALKWILNTIGQGIDWDKMYGFQCMDLVVAYLYYVTDGKIAMWGNAIDAPKNNFKGTAKVIKNYPAFRPEEGDIVVWSYGNFSTYGHIAVVIDGDPYGDLQYITVAEQNWNGLGLYKQEVTTKRIHNYDGVSHFIRPKFKKTSNSTSSSNNNGAAQSNHSASWLNNYKKGYGYGPYPLGINGGNHYGVDFFMNVGTPVRAISDGKIVEAGWTNYGGGNEIGLVENDGVHRQWYMHLSKFNVKVGDRVKAGQIIGWSGSTGYSTAPHLHFQRMTNSFSNNTAQDPMPFLKSAGYGSNSTSSSNNNGYKTNKYGTLYKSESASFTANTDIITRLTGPFRSMPQSGVLRKGLTIKYDEVMKQDGHVWVGYNTNSGKRVYLPVRTWNESTGELGPLWGTIK

SEQ ID NO: 32 - protein, 402 aa, Artificial Sequence
  CHAPSEP_M23Ale1_SH3bLST
MKTKKQALKWILNTIGQGIDWDKMYGFQCMDLVVAYLYYVTDGKIAMWGNAIDAPKNNFKGTAKVIKNYPAFRPEEGDIVVWSYGNFSTYGHIAVVIDGDPYGDLQYITVAEQNWNGLGLYKQEVTTKRIHNYDGVSHFIRPKFKKTSNSTSSSNNNGAAQSNHSASWLNNYKKGYGYGPYPLGINGGNHYGVDFFMNVGTPVRAISDGKIVEAGWTNYGGGNEIGLVENDGVHRQWYMHLSKFNVKVGDRVKAGQIIGWSGSTGYSTAPHLHFQRMTNSFSNNTAQDPMPFLKSAGYGSNSTSSSNNNGWKTNKYGTLYKSESASFTPNTDIITRTTGPFRSMPQSGVLKAGQTIHYDEVMKQDGHVWVGYTGNSGQRIYLPVRTWNKSTNTLGVLWGTIK

SEQ ID NO: 33 - protein, 404 aa, Artificial Sequence
  CHAPSEP_M23LST_SH3b2638
MKTKKQALKWILNTIGQGIDWDKMYGFQCMDLVVAYLYYVTDGKIAMWGNAIDAPKNNFKGTAKVIKNYPAFRPEEGDIVVWSYGNFSTYGHIAVVIDGDPYGDLQYITVAEQNWNGLGLYKQEVTTKRIHNYDGVSHFIRPKFKKTSNSTSSSNNNGAATHEHSAQWLNNYKKGYGYGPYPLGINGGMHYGVDFFMNIGTPVKAISSGKIVEAGWSNYGGGNQIGLIENDGVHRQWYMHLSKYNVKVGDYVKAGQIIGWSGSTGYSTAPHLHFQRMVNSFSNSTAQDPMPFLKSAGYGSNSTSSSNNNGWKQNKDGIWYKAEHASFTVTAPEGIITRYKGPWTGHPQAGVLQKGQTIKYDEVQKFDGHVWVSWETFEGETVYMPVRTWDAKTGKVGKLWGEIK

SEQ ID NO: 34 - protein, 402 aa, Artificial Sequence
  CHAPSEP_M23LST_SH3bAle1
MKTKKQALKWILNTIGQGIDWDKMYGFQCMDLVVAYLYYVTDGKIAMWGNAIDAPKNNFKGTAKVIKNYPAFRPEEGDIVVWSYGNFSTYGHIAVVIDGDPYGDLQYITVAEQNWNGLGLYKQEVTTKRIHNYDGVSHFIRPKFKKTSNSTSSSNNNGAATHEHSAQWLNNYKKGYGYGPYPLGINGGMHYGVDFFMNIGTPVKAISSGKIVEAGWSNYGGGNQIGLIENDGVHRQWYMHLSKYNVKVGDYVKAGQIIGWSGSTGYSTAPHLHFQRMVNSFSNSTAQDPMPFLKSAGYGSNSTSSSNNNGYKTNKYGTLYKSESASFTANTDIITRLTGPFRSMPQSGVLRKGLTIKYDEVMKQDGHVWVGYNTNSGKRVYLPVRTWNESTGELGPLWGTIK

SEQ ID NO: 35 - protein, 402 aa, Artificial Sequence
  CHAPSEP_M23LST_SH3bLST
MKTKKQALKWILNTIGQGIDWDKMYGFQCMDLVVAYLYYVTDGKIAMWGNAIDAPKNNFKGTAKVIKNYPAFRPEEGDIVVWSYGNFSTYGHIAVVIDGDPYGDLQYITVAEQNWNGLGLYKQEVTTKRIHNYDGVSHFIRPKFKKTSNSTSSSNNNGAATHEHSAQWLNNYKKGYGYGPYPLGINGGMHYGVDFFMNIGTPVKAISSGKIVEAGWSNYGGGNQIGLIENDGVHRQWYMHLSKYNVKVGDYVKAGQIIGWSGSTGYSTAPHLHFQRMVNSFSNSTAQDPMPFLKSAGYGSNSTSSSNNNGWKTNKYGTLYKSESASFTPNTDIITRTTGPFRSMPQSGVLKAGQTIHYDEVMKQDGHVWVGYTGNSGQRIYLPVRTWNKSTNTLGVLWGTIK

SEQ ID NO: 36 - protein, 404 aa, Artificial Sequence
  CHAPTw_M23Ale1_SH3b2638
KTLKQAESYIKSKVNTGTDFDGLYGYQCMDLAVDYIYHVTDGKIRMWGNAKDAINNSFGGTATVYKNYPAFRPKYGDVVVWTTGNFATYGHIAIVTNPDPYGDLQYVTVLEQNWNGNGIYKTELATIRTHDYTGITHFIRPNFATESSNSTSSSNNNGAAQSNHSASWLNNYKKGYGYGPYPLGINGGNHYGVDFFMNVGTPVRAISDGKIVEAGWTNYGGGNEIGLVENDGVHRQWYMHLSKFNVKVGDRVKAGQIIGWSGSTGYSTAPHLHFQRMTNSFSNNTAQDPMPFLKSAGYGSNSTSSSNNNGWKQNKDGIWYKAEHASFTVTAPEGIITRYKGPWTGHPQAGVLQKGQTIKYDEVQKFDGHVWVSWETFEGETVYMPVRTWDAKTGKVGKLWGEIK

SEQ ID NO: 37 - protein, 402 aa, Artificial Sequence
  CHAPTw_M23Ale1_SH3bAle1
KTLKQAESYIKSKVNTGTDFDGLYGYQCMDLAVDYIYHVTDGKIRMWGNAKDAINNSFGGTATVYKNYPAFRPKYGDVVVWTTGNFATYGHIAIVTNPDPYGDLQYVTVLEQNWNGNGIYKTELATIRTHDYTGITHFIRPNFATESSNSTSSSNNNGAAQSNHSASWLNNYKKGYGYGPYPLGINGGNHYGVDFFMNVGTPVRAISDGKIVEAGWTNYGGGNEIGLVENDGVHRQWYMHLSKFNVKVGDRVKAGQIIGWSGSTGYSTAPHLHFQRMTNSFSNNTAQDPMPFLKSAGYGSNSTSSSNNNGYKTNKYGTLYKSESASFTANTDIITRLTGPFRSMPQSGVLRKGLTIKYDEVMKQDGHVWVGYNTNSGKRVYLPVRTWNESTGELGPLWGTIK

SEQ ID NO: 38 - protein, 402 aa, Artificial Sequence
  CHAPTw_M23Ale1_SH3bLST
KTLKQAESYIKSKVNTGTDFDGLYGYQCMDLAVDYIYHVTDGKIRMWGNAKDAINNSFGGTATVYKNYPAFRPKYGDVVVWTTGNFATYGHIAIVTNPDPYGDLQYVTVLEQNWNGNGIYKTELATIRTHDYTGITHFIRPNFATESSNSTSSSNNNGAAQSNHSASWLNNYKKGYGYGPYPLGINGGNHYGVDFFMNVGTPVRAISDGKIVEAGWTNYGGGNEIGLVENDGVHRQWYMHLSKFNVKVGDRVKAGQIIGWSGSTGYSTAPHLHFQRMTNSFSNNTAQDPMPFLKSAGYGSNSTSSSNNNGWKTNKYGTLYKSESASFTPNTDIITRTTGPFRSMPQSGVLKAGQTIHYDEVMKQDGHVWVGYTGNSGQRIYLPVRTWNKSTNTLGVLWGTIK

SEQ ID NO: 39 - protein, 404 aa, Artificial Sequence
  CHAPTw_M23LST_SH3b2638
KTLKQAESYIKSKVNTGTDFDGLYGYQCMDLAVDYIYHVTDGKIRMWGNAKDAINNSFGGTATVYKNYPAFRPKYGDVVVWTTGNFATYGHIAIVTNPDPYGDLQYVTVLEQNWNGNGIYKTELATIRTHDYTGITHFIRPNFATESSNSTSSSNNNGAATHEHSAQWLNNYKKGYGYGPYPLGINGGMHYGVDFFMNIGTPVKAISSGKIVEAGWSNYGGGNQIGLIENDGVHRQWYMHLSKYNVKVGDYVKAGQIIGWSGSTGYSTAPHLHFQRMVNSFSNSTAQDPMPFLKSAGYGSNSTSSSNNNGWKQNKDGIWYKAEHASFTVTAPEGIITRYKGPWTGHPQAGVLQKGQTIKYDEVQKFDGHVWVSWETFEGETVYMPVRTWDAKTGKVGKLWGEIK

SEQ ID NO: 40 - protein, 402 aa, Artificial Sequence
  CHAPTw_M23LST_ SH3bAle1
KTLKQAESYIKSKVNTGTDFDGLYGYQCMDLAVDYIYHVTDGKIRMWGNAKDAINNSFGGTATVYKNYPAFRPKYGDVVVWTTGNFATYGHIAIVTNPDPYGDLQYVTVLEQNWNGNGIYKTELATIRTHDYTGITHFIRPNFATESSNSTSSSNNNGAATHEHSAQWLNNYKKGYGYGPYPLGINGGMHYGVDFFMNIGTPVKAISSGKIVEAGWSNYGGGNQIGLIENDGVHRQWYMHLSKYNVKVGDYVKAGQIIGWSGSTGYSTAPHLHFQRMVNSFSNSTAQDPMPFLKSAGYGSNSTSSSNNNGYKTNKYGTLYKSESASFTANTDIITRLTGPFRSMPQSGVLRKGLTIKYDEVMKQDGHVWVGYNTNSGKRVYLPVRTWNESTGELGPLWGTIK

SEQ ID NO: 41 - protein, 402 aa, Artificial Sequence
  CHAPTw_M23LST_SH3bLST
KTLKQAESYIKSKVNTGTDFDGLYGYQCMDLAVDYIYHVTDGKIRMWGNAKDAINNSFGGTATVYKNYPAFRPKYGDVVVWTTGNFATYGHIAIVTNPDPYGDLQYVTVLEQNWNGNGIYKTELATIRTHDYTGITHFIRPNFATESSNSTSSSNNNGAATHEHSAQWLNNYKKGYGYGPYPLGINGGMHYGVDFFMNIGTPVKAISSGKIVEAGWSNYGGGNQIGLIENDGVHRQWYMHLSKYNVKVGDYVKAGQIIGWSGSTGYSTAPHLHFQRMVNSFSNSTAQDPMPFLKSAGYGSNSTSSSNNNGWKTNKYGTLYKSESASFTPNTDIITRTTGPFRSMPQSGVLKAGQTIHYDEVMKQDGHVWVGYTGNSGQRIYLPVRTWNKSTNTLGVLWGTIK

SEQ ID NO: 42 - protein, 394 aa, Artificial Sequence
  TCHAPK_M23Ale1_SH3b2638
SLKKYNGKLPKHDPSFVQPGNRHYKYQCTWYAYNRRGQLGIPVPLWGDAADWIGGAKGAGYGVGRTPKQGACVIWQRGVQGGSPQYGHVAFVEKVLDGGKKIFISEHNYATPNGYGTRTIDMSSAIGKNAQFIYDKKSNSTSSSNNNGAAQSNHSASWLNNYKKGYGYGPYPLGINGGNHYGVDFFMNVGTPVRAISDGKIVEAGWTNYGGGNEIGLVENDGVHRQWYMHLSKFNVKVGDRVKAGQIIGWSGSTGYSTAPHLHFQRMTNSFSNNTAQDPMPFLKSAGYGSNSTSSSNNNGWKQNKDGIWYKAEHASFTVTAPEGIITRYKGPWTGHPQAGVLQKGQTIKYDEVQKFDGHVWVSWETFEGETVYMPVRTWDAKTGKVGKLWGEIK

SEQ ID NO: 43 - protein, 392 aa, Artificial Sequence
  TCHAPK_M23Ale1_SH3bAle1
SLKKYNGKLPKHDPSFVQPGNRHYKYQCTWYAYNRRGQLGIPVPLWGDAADWIGGAKGAGYGVGRTPKQGACVIWQRGVQGGSPQYGHVAFVEKVLDGGKKIFISEHNYATPNGYGTRTIDMSSAIGKNAQFIYDKKSNSTSSSNNNGAAQSNHSASWLNNYKKGYGYGPYPLGINGGNHYGVDFFMNVGTPVRAISDGKIVEAGWTNYGGGNEIGLVENDGVHRQWYMHLSKFNVKVGDRVKAGQIIGWSGSTGYSTAPHLHFQRMTNSFSNNTAQDPMPFLKSAGYGSNSTSSSNNNGYKTNKYGTLYKSESASFTANTDIITRLTGPFRSMPQSGVLRKGLTIKYDEVMKQDGHVWVGYNTNSGKRVYLPVRTWNESTGELGPLWGTIK

SEQ ID NO: 44 - protein, 392 aa, Artificial Sequence
  TCHAPK_M23Ale1_SH3bLST
SLKKYNGKLPKHDPSFVQPGNRHYKYQCTWYAYNRRGQLGIPVPLWGDAADWIGGAKGAGYGVGRTPKQGACVIWQRGVQGGSPQYGHVAFVEKVLDGGKKIFISEHNYATPNGYGTRTIDMSSAIGKNAQFIYDKKSNSTSSSNNNGAAQSNHSASWLNNYKKGYGYGPYPLGINGGNHYGVDFFMNVGTPVRAISDGKIVEAGWTNYGGGNEIGLVENDGVHRQWYMHLSKFNVKVGDRVKAGQIIGWSGSTGYSTAPHLHFQRMTNSFSNNTAQDPMPFLKSAGYGSNSTSSSNNNGWKTNKYGTLYKSESASFTPNTDIITRTTGPFRSMPQSGVLKAGQTIHYDEVMKQDGHVWVGYTGNSGQRIYLPVRTWNKSTNTLGVLWGTIK

SEQ ID NO: 45 - protein, 394 aa, Artificial Sequence
  TCHAPK_M23LST_SH3b2638
SLKKYNGKLPKHDPSFVQPGNRHYKYQCTWYAYNRRGQLGIPVPLWGDAADWIGGAKGAGYGVGRTPKQGACVIWQRGVQGGSPQYGHVAFVEKVLDGGKKIFISEHNYATPNGYGTRTIDMSSAIGKNAQFIYDKKSNSTSSSNNNGAATHEHSAQWLNNYKKGYGYGPYPLGINGGMHYGVDFFMNIGTPVKAISSGKIVEAGWSNYGGGNQIGLIENDGVHRQWYMHLSKYNVKVGDYVKAGQIIGWSGSTGYSTAPHLHFQRMVNSFSNSTAQDPMPFLKSAGYGSNSTSSSNNNGWKQNKDGIWYKAEHASFTVTAPEGIITRYKGPWTGHPQAGVLQKGQTIKYDEVQKFDGHVWVSWETFEGETVYMPVRTWDAKTGKVGKLWGEIK

SEQ ID NO: 46 - protein, 392 aa, Artificial Sequence
  TCHAPK_M23LST_SH3bAle1
SLKKYNGKLPKHDPSFVQPGNRHYKYQCTWYAYNRRGQLGIPVPLWGDAADWIGGAKGAGYGVGRTPKQGACVIWQRGVQGGSPQYGHVAFVEKVLDGGKKIFISEHNYATPNGYGTRTIDMSSAIGKNAQFIYDKKSNSTSSSNNNGAATHEHSAQWLNNYKKGYGYGPYPLGINGGMHYGVDFFMNIGTPVKAISSGKIVEAGWSNYGGGNQIGLIENDGVHRQWYMHLSKYNVKVGDYVKAGQIIGWSGSTGYSTAPHLHFQRMVNSFSNSTAQDPMPFLKSAGYGSNSTSSSNNNGYKTNKYGTLYKSESASFTANTDIITRLTGPFRSMPQSGVLRKGLTIKYDEVMKQDGHVWVGYNTNSGKRVYLPVRTWNESTGELGPLWGTIK

SEQ ID NO: 47 - protein, 392 aa, Artificial Sequence
  TCHAPK_M23LST_SH3bLST
SLKKYNGKLPKHDPSFVQPGNRHYKYQCTWYAYNRRGQLGIPVPLWGDAADWIGGAKGAGYGVGRTPKQGACVIWQRGVQGGSPQYGHVAFVEKVLDGGKKIFISEHNYATPNGYGTRTIDMSSAIGKNAQFIYDKKSNSTSSSNNNGAATHEHSAQWLNNYKKGYGYGPYPLGINGGMHYGVDFFMNIGTPVKAISSGKIVEAGWSNYGGGNQIGLIENDGVHRQWYMHLSKYNVKVGDYVKAGQIIGWSGSTGYSTAPHLHFQRMVNSFSNSTAQDPMPFLKSAGYGSNSTSSSNNNGWKTNKYGTLYKSESASFTPNTDIITRTTGPFRSMPQSGVLKAGQTIHYDEVMKQDGHVWVGYTGNSGQRIYLPVRTWNKSTNTLGVLWGTIK

SEQ ID NO: 48 - protein, 392 aa, Artificial Sequence
  TCHAPTw_M23Ale1_SH3b2638
GKELPTPRNKTDTSWTAPGNPNTGQWARECTWYCYNRRYELGLKAVAYGDAADWIAGARGAGISTGKEPKRGAVAVWARGVPGGSAQYGHVAFVEKVTDDGIYVSDYNYASPKTYGERLYKKGSPEYRNAQYIYDSNSTSSSNNNGAAQSNHSASWLNNYKKGYGYGPYPLGINGGNHYGVDFFMNVGTPVRAISDGKIVEAGWTNYGGGNEIGLVENDGVHRQWYMHLSKFNVKVGDRVKAGQIIGWSGSTGYSTAPHLHFQRMTNSFSNNTAQDPMPFLKSAGYGSNSTSSSNNNGWKQNKDGIWYKAEHASFTVTAPEGIITRYKGPWTGHPQAGVLQKGQTIKYDEVQKFDGHVWVSWETFEGETVYMPVRTWDAKTGKVGKLWGEIK

SEQ ID NO: 49 - protein, 390 aa, Artificial Sequence
  TCHAPTw_M23Ale1_SH3bAle1
GKELPTPRNKTDTSWTAPGNPNTGQWARECTWYCYNRRYELGLKAVAYGDAADWIAGARGAGISTGKEPKRGAVAVWARGVPGGSAQYGHVAFVEKVTDDGIYVSDYNYASPKTYGERLYKKGSPEYRNAQYIYDSNSTSSSNNNGAAQSNHSASWLNNYKKGYGYGPYPLGINGGNHYGVDFFMNVGTPVRAISDGKIVEAGWTNYGGGNEIGLVENDGVHRQWYMHLSKFNVKVGDRVKAGQIIGWSGSTGYSTAPHLHFQRMTNSFSNNTAQDPMPFLKSAGYGSNSTSSSNNNGYKTNKYGTLYKSESASFTANTDIITRLTGPFRSMPQSGVLRKGLTIKYDEVMKQDGHVWVGYNTNSGKRVYLPVRTWNESTGELGPLWGTIK

SEQ ID NO: 50 - protein, 390 aa, Artificial Sequence
  TCHAPTw_M23Ale1_SH3bLST
GKELPTPRNKTDTSWTAPGNPNTGQWARECTWYCYNRRYELGLKAVAYGDAADWIAGARGAGISTGKEPKRGAVAVWARGVPGGSAQYGHVAFVEKVTDDGIYVSDYNYASPKTYGERLYKKGSPEYRNAQYIYDSNSTSSSNNNGAAQSNHSASWLNNYKKGYGYGPYPLGINGGNHYGVDFFMNVGTPVRAISDGKIVEAGWTNYGGGNEIGLVENDGVHRQWYMHLSKFNVKVGDRVKAGQIIGWSGSTGYSTAPHLHFQRMTNSFSNNTAQDPMPFLKSAGYGSNSTSSSNNNGWKTNKYGTLYKSESASFTPNTDIITRTTGPFRSMPQSGVLKAGQTIHYDEVMKQDGHVWVGYTGNSGQRIYLPVRTWNKSTNTLGVLWGTIK

SEQ ID NO: 51 - protein, 392 aa, Artificial Sequence
  TCHAPTw_M23LST_SH3b2638
GKELPTPRNKTDTSWTAPGNPNTGQWARECTWYCYNRRYELGLKAVAYGDAADWIAGARGAGISTGKEPKRGAVAVWARGVPGGSAQYGHVAFVEKVTDDGIYVSDYNYASPKTYGERLYKKGSPEYRNAQYIYDSNSTSSSNNNGAATHEHSAQWLNNYKKGYGYGPYPLGINGGMHYGVDFFMNIGTPVKAISSGKIVEAGWSNYGGGNQIGLIENDGVHRQWYMHLSKYNVKVGDYVKAGQIIGWSGSTGYSTAPHLHFQRMVNSFSNSTAQDPMPFLKSAGYGSNSTSSSNNNGWKQNKDGIWYKAEHASFTVTAPEGIITRYKGPWTGHPQAGVLQKGQTIKYDEVQKFDGHVWVSWETFEGETVYMPVRTWDAKTGKVGKLWGEIK

SEQ ID NO: 52 - protein, 390 aa, Artificial Sequence
  TCHAPTw_M23LST_SH3bAle1
GKELPTPRNKTDTSWTAPGNPNTGQWARECTWYCYNRRYELGLKAVAYGDAADWIAGARGAGISTGKEPKRGAVAVWARGVPGGSAQYGHVAFVEKVTDDGIYVSDYNYASPKTYGERLYKKGSPEYRNAQYIYDSNSTSSSNNNGAATHEHSAQWLNNYKKGYGYGPYPLGINGGMHYGVDFFMNIGTPVKAISSGKIVEAGWSNYGGGNQIGLIENDGVHRQWYMHLSKYNVKVGDYVKAGQIIGWSGSTGYSTAPHLHFQRMVNSFSNSTAQDPMPFLKSAGYGSNSTSSSNNNGYKTNKYGTLYKSESASFTANTDIITRLTGPFRSMPQSGVLRKGLTIKYDEVMKQDGHVWVGYNTNSGKRVYLPVRTWNESTGELGPLWGTIK

SEQ ID NO: 53 - protein, 390 aa, Artificial Sequence
  TCHAPTw_M23LST_SH3bLST
GKELPTPRNKTDTSWTAPGNPNTGQWARECTWYCYNRRYELGLKAVAYGDAADWIAGARGAGISTGKEPKRGAVAVWARGVPGGSAQYGHVAFVEKVTDDGIYVSDYNYASPKTYGERLYKKGSPEYRNAQYIYDSNSTSSSNNNGAATHEHSAQWLNNYKKGYGYGPYPLGINGGMHYGVDFFMNIGTPVKAISSGKIVEAGWSNYGGGNQIGLIENDGVHRQWYMHLSKYNVKVGDYVKAGQIIGWSGSTGYSTAPHLHFQRMVNSFSNSTAQDPMPFLKSAGYGSNSTSSSNNNGWKTNKYGTLYKSESASFTPNTDIITRTTGPFRSMPQSGVLKAGQTIHYDEVMKQDGHVWVGYTGNSGQRIYLPVRTWNKSTNTLGVLWGTIK

SEQ ID NO: 54 - protein, 422 aa, Artificial Sequence
  M23Ale1_CHAPGH15_SH3b2638
AAQSNHSASWLNNYKKGYGYGPYPLGINGGNHYGVDFFMNVGTPVRAISDGKIVEAGWTNYGGGNEIGLVENDGVHRQWYMHLSKFNVKVGDRVKAGQIIGWSGSTGYSTAPHLHFQRMTNSFSNNTAQDPMPFLKSAGYGSNSTSSSNNNGAKTQAEINKRLDAYAKGTVDSPYRIKKATSYDPSFGVMEAGAIDADGYYHAQCQDLITDYVLWLTDNKVRTWGNAKDQIKQSYGTGFKIHENKPSTVPKKGWIAVFTSGSYQQWGHIGIVYDGGNTSTFTILEQNWNGYANKKPTKRVDNYYGLTHFIEIPVKAGSNSTSSSNNNGWKQNKDGIWYKAEHASFTVTAPEGIITRYKGPWTGHPQAGVLQKGQTIKYDEVQKFDGHVWVSWETFEGETVYMPVRTWDAKTGKVGKLWGEIK

SEQ ID NO: 55 - protein, 420 aa, Artificial Sequence
  M23Ale1_CHAPGH15_SH3bAle1
AAQSNHSASWLNNYKKGYGYGPYPLGINGGNHYGVDFFMNVGTPVRAISDGKIVEAGWTNYGGGNEIGLVENDGVHRQWYMHLSKFNVKVGDRVKAGQIIGWSGSTGYSTAPHLHFQRMTNSFSNNTAQDPMPFLKSAGYGSNSTSSSNNNGAKTQAEINKRLDAYAKGTVDSPYRIKKATSYDPSFGVMEAGAIDADGYYHAQCQDLITDYVLWLTDNKVRTWGNAKDQIKQSYGTGFKIHENKPSTVPKKGWIAVFTSGSYQQWGHIGIVYDGGNTSTFTILEQNWNGYANKKPTKRVDNYYGLTHFIEIPVKAGSNSTSSSNNNGYKTNKYGTLYKSESASFTANTDIITRLTGPFRSMPQSGVLRKGLTIKYDEVMKQDGHVWVGYNTNSGKRVYLPVRTWNESTGELGPLWGTIK

SEQ ID NO: 56 - protein, 420 aa, Artificial Sequence
  M23Ale1_CHAPGH15_SH3bLST
AAQSNHSASWLNNYKKGYGYGPYPLGINGGNHYGVDFFMNVGTPVRAISDGKIVEAGWTNYGGGNEIGLVENDGVHRQWYMHLSKFNVKVGDRVKAGQIIGWSGSTGYSTAPHLHFQRMTNSFSNNTAQDPMPFLKSAGYGSNSTSSSNNNGAKTQAEINKRLDAYAKGTVDSPYRIKKATSYDPSFGVMEAGAIDADGYYHAQCQDLITDYVLWLTDNKVRTWGNAKDQIKQSYGTGFKIHENKPSTVPKKGWIAVFTSGSYQQWGHIGIVYDGGNTSTFTILEQNWNGYANKKPTKRVDNYYGLTHFIEIPVKAGSNSTSSSNNNGWKTNKYGTLYKSESASFTPNTDIITRTTGPFRSMPQSGVLKAGQTIHYDEVMKQDGHVWVGYTGNSGQRIYLPVRTWNKSTNTLGVLWGTIK

SEQ ID NO: 57 - protein, 404 aa, Artificial Sequence
  M23Ale1_CHAPSEP_SH3b2638
AAQSNHSASWLNNYKKGYGYGPYPLGINGGNHYGVDFFMNVGTPVRAISDGKIVEAGWTNYGGGNEIGLVENDGVHRQWYMHLSKFNVKVGDRVKAGQIIGWSGSTGYSTAPHLHFQRMTNSFSNNTAQDPMPFLKSAGYGSNSTSSSNNNGMKTKKQALKWILNTIGQGIDWDKMYGFQCMDLVVAYLYYVTDGKIAMWGNAIDAPKNNFKGTAKVIKNYPAFRPEEGDIVVWSYGNFSTYGHIAVVIDGDPYGDLQYITVAEQNWNGLGLYKQEVTTKRIHNYDGVSHFIRPKFKKTSNSTSSSNNNGWKQNKDGIWYKAEHASFTVTAPEGIITRYKGPWTGHPQAGVLQKGQTIKYDEVQKFDGHVWVSWETFEGETVYMPVRTWDAKTGKVGKLWGEIK

SEQ ID NO: 58 - protein, 402 aa, Artificial Sequence
  M23Ale1_CHAPSEP_SH3bAle1
AAQSNHSASWLNNYKKGYGYGPYPLGINGGNHYGVDFFMNVGTPVRAISDGKIVEAGWTNYGGGNEIGLVENDGVHRQWYMHLSKFNVKVGDRVKAGQIIGWSGSTGYSTAPHLHFQRMTNSFSNNTAQDPMPFLKSAGYGSNSTSSSNNNGMKTKKQALKWILNTIGQGIDWDKMYGFQCMDLVVAYLYYVTDGKIAMWGNAIDAPKNNFKGTAKVIKNYPAFRPEEGDIVVWSYGNFSTYGHIAVVIDGDPYGDLQYITVAEQNWNGLGLYKQEVTTKRIHNYDGVSHFIRPKFKKTSNSTSSSNNNGYKTNKYGTLYKSESASFTANTDIITRLTGPFRSMPQSGVLRKGLTIKYDEVMKQDGHVWVGYNTNSGKRVYLPVRTWNESTGELGPLWGTIK

SEQ ID NO: 59 - protein, 402 aa, Artificial Sequence
  M23Ale1_CHAPSEP_SH3bLST
AAQSNHSASWLNNYKKGYGYGPYPLGINGGNHYGVDFFMNVGTPVRAISDGKIVEAGWTNYGGGNEIGLVENDGVHRQWYMHLSKFNVKVGDRVKAGQIIGWSGSTGYSTAPHLHFQRMTNSFSNNTAQDPMPFLKSAGYGSNSTSSSNNNGMKTKKQALKWILNTIGQGIDWDKMYGFQCMDLVVAYLYYVTDGKIAMWGNAIDAPKNNFKGTAKVIKNYPAFRPEEGDIVVWSYGNFSTYGHIAVVIDGDPYGDLQYITVAEQNWNGLGLYKQEVTTKRIHNYDGVSHFIRPKFKKTSNSTSSSNNNGWKTNKYGTLYKSESASFTPNTDIITRTTGPFRSMPQSGVLKAGQTIHYDEVMKQDGHVWVGYTGNSGQRIYLPVRTWNKSTNTLGVLWGTIK

SEQ ID NO: 60 - protein, 404 aa, Artificial Sequence
  M23Ale1_CHAPTw_SH3b2638
AAQSNHSASWLNNYKKGYGYGPYPLGINGGNHYGVDFFMNVGTPVRAISDGKIVEAGWTNYGGGNEIGLVENDGVHRQWYMHLSKFNVKVGDRVKAGQIIGWSGSTGYSTAPHLHFQRMTNSFSNNTAQDPMPFLKSAGYGSNSTSSSNNNGKTLKQAESYIKSKVNTGTDFDGLYGYQCMDLAVDYIYHVTDGKIRMWGNAKDAINNSFGGTATVYKNYPAFRPKYGDVVVWTTGNFATYGHIAIVTNPDPYGDLQYVTVLEQNWNGNGIYKTELATIRTHDYTGITHFIRPNFATESSNSTSSSNNNGWKQNKDGIWYKAEHASFTVTAPEGIITRYKGPWTGHPQAGVLQKGQTIKYDEVQKFDGHVWVSWETFEGETVYMPVRTWDAKTGKVGKLWGEIK

SEQ ID NO: 61 - protein, 402 aa, Artificial Sequence
  M23Ale1_CHAPTw_SH3bAle1
AAQSNHSASWLNNYKKGYGYGPYPLGINGGNHYGVDFFMNVGTPVRAISDGKIVEAGWTNYGGGNEIGLVENDGVHRQWYMHLSKFNVKVGDRVKAGQIIGWSGSTGYSTAPHLHFQRMTNSFSNNTAQDPMPFLKSAGYGSNSTSSSNNNGKTLKQAESYIKSKVNTGTDFDGLYGYQCMDLAVDYIYHVTDGKIRMWGNAKDAINNSFGGTATVYKNYPAFRPKYGDVVVWTTGNFATYGHIAIVTNPDPYGDLQYVTVLEQNWNGNGIYKTELATIRTHDYTGITHFIRPNFATESSNSTSSSNNNGYKTNKYGTLYKSESASFTANTDIITRLTGPFRSMPQSGVLRKGLTIKYDEVMKQDGHVWVGYNTNSGKRVYLPVRTWNESTGELGPLWGTIK

SEQ ID NO: 62 - protein, 402 aa, Artificial Sequence
  M23Ale1_CHAPTw_SH3bLST
AAQSNHSASWLNNYKKGYGYGPYPLGINGGNHYGVDFFMNVGTPVRAISDGKIVEAGWTNYGGGNEIGLVENDGVHRQWYMHLSKFNVKVGDRVKAGQIIGWSGSTGYSTAPHLHFQRMTNSFSNNTAQDPMPFLKSAGYGSNSTSSSNNNGKTLKQAESYIKSKVNTGTDFDGLYGYQCMDLAVDYIYHVTDGKIRMWGNAKDAINNSFGGTATVYKNYPAFRPKYGDVVVWTTGNFATYGHIAIVTNPDPYGDLQYVTVLEQNWNGNGIYKTELATIRTHDYTGITHFIRPNFATESSNSTSSSNNNGWKTNKYGTLYKSESASFTPNTDIITRTTGPFRSMPQSGVLKAGQTIHYDEVMKQDGHVWVGYTGNSGQRIYLPVRTWNKSTNTLGVLWGTIK

SEQ ID NO: 63 - protein, 394 aa, Artificial Sequence
  M23Ale1_TCHAPK_SH3b2638
AAQSNHSASWLNNYKKGYGYGPYPLGINGGNHYGVDFFMNVGTPVRAISDGKIVEAGWTNYGGGNEIGLVENDGVHRQWYMHLSKFNVKVGDRVKAGQIIGWSGSTGYSTAPHLHFQRMTNSFSNNTAQDPMPFLKSAGYGSNSTSSSNNNGSLKKYNGKLPKHDPSFVQPGNRHYKYQCTWYAYNRRGQLGIPVPLWGDAADWIGGAKGAGYGVGRTPKQGACVIWQRGVQGGSPQYGHVAFVEKVLDGGKKIFISEHNYATPNGYGTRTIDMSSAIGKNAQFIYDKKSNSTSSSNNNGWKQNKDGIWYKAEHASFTVTAPEGIITRYKGPWTGHPQAGVLQKGQTIKYDEVQKFDGHVWVSWETFEGETVYMPVRTWDAKTGKVGKLWGEIK

SEQ ID NO: 64 - protein, 392 aa, Artificial Sequence
  M23Ale1_TCHAPK_SH3bAle1
AAQSNHSASWLNNYKKGYGYGPYPLGINGGNHYGVDFFMNVGTPVRAISDGKIVEAGWTNYGGGNEIGLVENDGVHRQWYMHLSKFNVKVGDRVKAGQIIGWSGSTGYSTAPHLHFQRMTNSFSNNTAQDPMPFLKSAGYGSNSTSSSNNNGSLKKYNGKLPKHDPSFVQPGNRHYKYQCTWYAYNRRGQLGIPVPLWGDAADWIGGAKGAGYGVGRTPKQGACVIWQRGVQGGSPQYGHVAFVEKVLDGGKKIFISEHNYATPNGYGTRTIDMSSAIGKNAQFIYDKKSNSTSSSNNNGYKTNKYGTLYKSESASFTANTDIITRLTGPFRSMPQSGVLRKGLTIKYDEVMKQDGHVWVGYNTNSGKRVYLPVRTWNESTGELGPLWGTIK

SEQ ID NO: 65 - protein, 392 aa, Artificial Sequence
  M23Ale1_TCHAPK_SH3bLST
AAQSNHSASWLNNYKKGYGYGPYPLGINGGNHYGVDFFMNVGTPVRAISDGKIVEAGWTNYGGGNEIGLVENDGVHRQWYMHLSKFNVKVGDRVKAGQIIGWSGSTGYSTAPHLHFQRMTNSFSNNTAQDPMPFLKSAGYGSNSTSSSNNNGSLKKYNGKLPKHDPSFVQPGNRHYKYQCTWYAYNRRGQLGIPVPLWGDAADWIGGAKGAGYGVGRTPKQGACVIWQRGVQGGSPQYGHVAFVEKVLDGGKKIFISEHNYATPNGYGTRTIDMSSAIGKNAQFIYDKKSNSTSSSNNNGWKTNKYGTLYKSESASFTPNTDIITRTTGPFRSMPQSGVLKAGQTIHYDEVMKQDGHVWVGYTGNSGQRIYLPVRTWNKSTNTLGVLWGTIK

SEQ ID NO: 66 - protein, 392 aa, Artificial Sequence
  M23Ale1_TCHAPTw_SH3b2638
AAQSNHSASWLNNYKKGYGYGPYPLGINGGNHYGVDFFMNVGTPVRAISDGKIVEAGWTNYGGGNEIGLVENDGVHRQWYMHLSKFNVKVGDRVKAGQIIGWSGSTGYSTAPHLHFQRMTNSFSNNTAQDPMPFLKSAGYGSNSTSSSNNNGGKELPTPRNKTDTSWTAPGNPNTGQWARECTWYCYNRRYELGLKAVAYGDAADWIAGARGAGISTGKEPKRGAVAVWARGVPGGSAQYGHVAFVEKVTDDGIYVSDYNYASPKTYGERLYKKGSPEYRNAQYIYDSNSTSSSNNNGWKQNKDGIWYKAEHASFTVTAPEGIITRYKGPWTGHPQAGVLQKGQTIKYDEVQKFDGHVWVSWETFEGETVYMPVRTWDAKTGKVGKLWGEIK

SEQ ID NO: 67 - protein, 390 aa, Artificial Sequence
  M23Ale1_TCHAPTw_SH3bAle1
AAQSNHSASWLNNYKKGYGYGPYPLGINGGNHYGVDFFMNVGTPVRAISDGKIVEAGWTNYGGGNEIGLVENDGVHRQWYMHLSKFNVKVGDRVKAGQIIGWSGSTGYSTAPHLHFQRMTNSFSNNTAQDPMPFLKSAGYGSNSTSSSNNNGGKELPTPRNKTDTSWTAPGNPNTGQWARECTWYCYNRRYELGLKAVAYGDAADWIAGARGAGISTGKEPKRGAVAVWARGVPGGSAQYGHVAFVEKVTDDGIYVSDYNYASPKTYGERLYKKGSPEYRNAQYIYDSNSTSSSNNNGYKTNKYGTLYKSESASFTANTDIITRLTGPFRSMPQSGVLRKGLTIKYDEVMKQDGHVWVGYNTNSGKRVYLPVRTWNESTGELGPLWGTIK

SEQ ID NO: 68 - protein, 390 aa, Artificial Sequence
  M23Ale1_TCHAPTw_SH3bLST
AAQSNHSASWLNNYKKGYGYGPYPLGINGGNHYGVDFFMNVGTPVRAISDGKIVEAGWTNYGGGNEIGLVENDGVHRQWYMHLSKFNVKVGDRVKAGQIIGWSGSTGYSTAPHLHFQRMTNSFSNNTAQDPMPFLKSAGYGSNSTSSSNNNGGKELPTPRNKTDTSWTAPGNPNTGQWARECTWYCYNRRYELGLKAVAYGDAADWIAGARGAGISTGKEPKRGAVAVWARGVPGGSAQYGHVAFVEKVTDDGIYVSDYNYASPKTYGERLYKKGSPEYRNAQYIYDSNSTSSSNNNGWKTNKYGTLYKSESASFTPNTDIITRTTGPFRSMPQSGVLKAGQTIHYDEVMKQDGHVWVGYTGNSGQRIYLPVRTWNKSTNTLGVLWGTIK

SEQ ID NO: 69 - protein, 422 aa, Artificial Sequence
  M23LST_CHAPGH15_SH3b2638
AATHEHSAQWLNNYKKGYGYGPYPLGINGGMHYGVDFFMNIGTPVKAISSGKIVEAGWSNYGGGNQIGLIENDGVHRQWYMHLSKYNVKVGDYVKAGQIIGWSGSTGYSTAPHLHFQRMVNSFSNSTAQDPMPFLKSAGYGSNSTSSSNNNGAKTQAEINKRLDAYAKGTVDSPYRIKKATSYDPSFGVMEAGAIDADGYYHAQCQDLITDYVLWLTDNKVRTWGNAKDQIKQSYGTGFKIHENKPSTVPKKGWIAVFTSGSYQQWGHIGIVYDGGNTSTFTILEQNWNGYANKKPTKRVDNYYGLTHFIEIPVKAGSNSTSSSNNNGWKQNKDGIWYKAEHASFTVTAPEGIITRYKGPWTGHPQAGVLQKGQTIKYDEVQKFDGHVWVSWETFEGETVYMPVRTWDAKTGKVGKLWGEIK

SEQ ID NO: 70 - protein, 420 aa, Artificial Sequence
  M23LST_CHAPGH15_SH3bAle1
AATHEHSAQWLNNYKKGYGYGPYPLGINGGMHYGVDFFMNIGTPVKAISSGKIVEAGWSNYGGGNQIGLIENDGVHRQWYMHLSKYNVKVGDYVKAGQIIGWSGSTGYSTAPHLHFQRMVNSFSNSTAQDPMPFLKSAGYGSNSTSSSNNNGAKTQAEINKRLDAYAKGTVDSPYRIKKATSYDPSFGVMEAGAIDADGYYHAQCQDLITDYVLWLTDNKVRTWGNAKDQIKQSYGTGFKIHENKPSTVPKKGWIAVFTSGSYQQWGHIGIVYDGGNTSTFTILEQNWNGYANKKPTKRVDNYYGLTHFIEIPVKAGSNSTSSSNNNGYKTNKYGTLYKSESASFTANTDIITRLTGPFRSMPQSGVLRKGLTIKYDEVMKQDGHVWVGYNTNSGKRVYLPVRTWNESTGELGPLWGTIK

SEQ ID NO: 71 - protein, 420 aa, Artificial Sequence
  M23LST_CHAPGH15_SH3bLST
AATHEHSAQWLNNYKKGYGYGPYPLGINGGMHYGVDFFMNIGTPVKAISSGKIVEAGWSNYGGGNQIGLIENDGVHRQWYMHLSKYNVKVGDYVKAGQIIGWSGSTGYSTAPHLHFQRMVNSFSNSTAQDPMPFLKSAGYGSNSTSSSNNNGAKTQAEINKRLDAYAKGTVDSPYRIKKATSYDPSFGVMEAGAIDADGYYHAQCQDLITDYVLWLTDNKVRTWGNAKDQIKQSYGTGFKIHENKPSTVPKKGWIAVFTSGSYQQWGHIGIVYDGGNTSTFTILEQNWNGYANKKPTKRVDNYYGLTHFIEIPVKAGSNSTSSSNNNGWKTNKYGTLYKSESASFTPNTDIITRTTGPFRSMPQSGVLKAGQTIHYDEVMKQDGHVWVGYTGNSGQRIYLPVRTWNKSTNTLGVLWGTIK

SEQ ID NO: 72 - protein, 404 aa, Artificial Sequence
  M23LST_CHAPSEP_SH3b2638
AATHEHSAQWLNNYKKGYGYGPYPLGINGGMHYGVDFFMNIGTPVKAISSGKIVEAGWSNYGGGNQIGLIENDGVHRQWYMHLSKYNVKVGDYVKAGQIIGWSGSTGYSTAPHLHFQRMVNSFSNSTAQDPMPFLKSAGYGSNSTSSSNNNGMKTKKQALKWILNTIGQGIDWDKMYGFQCMDLVVAYLYYVTDGKIAMWGNAIDAPKNNFKGTAKVIKNYPAFRPEEGDIVVWSYGNFSTYGHIAVVIDGDPYGDLQYITVAEQNWNGLGLYKQEVTTKRIHNYDGVSHFIRPKFKKTSNSTSSSNNNGWKQNKDGIWYKAEHASFTVTAPEGIITRYKGPWTGHPQAGVLQKGQTIKYDEVQKFDGHVWVSWETFEGETVYMPVRTWDAKTGKVGKLWGEIK

SEQ ID NO: 73 - protein, 402 aa, Artificial Sequence
  M23LST_CHAPSEP_SH3bAle1
AATHEHSAQWLNNYKKGYGYGPYPLGINGGMHYGVDFFMNIGTPVKAISSGKIVEAGWSNYGGGNQIGLIENDGVHRQWYMHLSKYNVKVGDYVKAGQIIGWSGSTGYSTAPHLHFQRMVNSFSNSTAQDPMPFLKSAGYGSNSTSSSNNNGMKTKKQALKWILNTIGQGIDWDKMYGFQCMDLVVAYLYYVTDGKIAMWGNAIDAPKNNFKGTAKVIKNYPAFRPEEGDIVVWSYGNFSTYGHIAVVIDGDPYGDLQYITVAEQNWNGLGLYKQEVTTKRIHNYDGVSHFIRPKFKKTSNSTSSSNNNGYKTNKYGTLYKSESASFTANTDIITRLTGPFRSMPQSGVLRKGLTIKYDEVMKQDGHVWVGYNTNSGKRVYLPVRTWNESTGELGPLWGTIK

SEQ ID NO: 74 - protein, 402 aa, Artificial Sequence
  M23LST_CHAPSEP_SH3bLST
AATHEHSAQWLNNYKKGYGYGPYPLGINGGMHYGVDFFMNIGTPVKAISSGKIVEAGWSNYGGGNQIGLIENDGVHRQWYMHLSKYNVKVGDYVKAGQIIGWSGSTGYSTAPHLHFQRMVNSFSNSTAQDPMPFLKSAGYGSNSTSSSNNNGMKTKKQALKWILNTIGQGIDWDKMYGFQCMDLVVAYLYYVTDGKIAMWGNAIDAPKNNFKGTAKVIKNYPAFRPEEGDIVVWSYGNFSTYGHIAVVIDGDPYGDLQYITVAEQNWNGLGLYKQEVTTKRIHNYDGVSHFIRPKFKKTSNSTSSSNNNGWKTNKYGTLYKSESASFTPNTDIITRTTGPFRSMPQSGVLKAGQTIHYDEVMKQDGHVWVGYTGNSGQRIYLPVRTWNKSTNTLGVLWGTIK

SEQ ID NO: 75 - protein, 402 aa, Artificial Sequence
  M23LST_CHAPTw__SH3bAle1
AATHEHSAQWLNNYKKGYGYGPYPLGINGGMHYGVDFFMNIGTPVKAISSGKIVEAGWSNYGGGNQIGLIENDGVHRQWYMHLSKYNVKVGDYVKAGQIIGWSGSTGYSTAPHLHFQRMVNSFSNSTAQDPMPFLKSAGYGSNSTSSSNNNGKTLKQAESYIKSKVNTGTDFDGLYGYQCMDLAVDYIYHVTDGKIRMWGNAKDAINNSFGGTATVYKNYPAFRPKYGDVVVWTTGNFATYGHIAIVTNPDPYGDLQYVTVLEQNWNGNGIYKTELATIRTHDYTGITHFIRPNFATESSNSTSSSNNNGYKTNKYGTLYKSESASFTANTDIITRLTGPFRSMPQSGVLRKGLTIKYDEVMKQDGHVWVGYNTNSGKRVYLPVRTWNESTGELGPLWGTIK

SEQ ID NO: 76 - protein, 404 aa, Artificial Sequence
  M23LST_CHAPTw_SH3b2638
AATHEHSAQWLNNYKKGYGYGPYPLGINGGMHYGVDFFMNIGTPVKAISSGKIVEAGWSNYGGGNQIGLIENDGVHRQWYMHLSKYNVKVGDYVKAGQIIGWSGSTGYSTAPHLHFQRMVNSFSNSTAQDPMPFLKSAGYGSNSTSSSNNNGKTLKQAESYIKSKVNTGTDFDGLYGYQCMDLAVDYIYHVTDGKIRMWGNAKDAINNSFGGTATVYKNYPAFRPKYGDVVVWTTGNFATYGHIAIVTNPDPYGDLQYVTVLEQNWNGNGIYKTELATIRTHDYTGITHFIRPNFATESSNSTSSSNNNGWKQNKDGIWYKAEHASFTVTAPEGIITRYKGPWTGHPQAGVLQKGQTIKYDEVQKFDGHVWVSWETFEGETVYMPVRTWDAKTGKVGKLWGEIK

SEQ ID NO: 77 - protein, 402 aa, Artificial Sequence
  M23LST_CHAPTw_SH3bLST
AATHEHSAQWLNNYKKGYGYGPYPLGINGGMHYGVDFFMNIGTPVKAISSGKIVEAGWSNYGGGNQIGLIENDGVHRQWYMHLSKYNVKVGDYVKAGQIIGWSGSTGYSTAPHLHFQRMVNSFSNSTAQDPMPFLKSAGYGSNSTSSSNNNGKTLKQAESYIKSKVNTGTDFDGLYGYQCMDLAVDYIYHVTDGKIRMWGNAKDAINNSFGGTATVYKNYPAFRPKYGDVVVWTTGNFATYGHIAIVTNPDPYGDLQYVTVLEQNWNGNGIYKTELATIRTHDYTGITHFIRPNFATESSNSTSSSNNNGWKTNKYGTLYKSESASFTPNTDIITRTTGPFRSMPQSGVLKAGQTIHYDEVMKQDGHVWVGYTGNSGQRIYLPVRTWNKSTNTLGVLWGTIK

SEQ ID NO: 78 - protein, 394 aa, Artificial Sequence
  M23LST_TCHAPK_SH3b2638
AATHEHSAQWLNNYKKGYGYGPYPLGINGGMHYGVDFFMNIGTPVKAISSGKIVEAGWSNYGGGNQIGLIENDGVHRQWYMHLSKYNVKVGDYVKAGQIIGWSGSTGYSTAPHLHFQRMVNSFSNSTAQDPMPFLKSAGYGSNSTSSSNNNGSLKKYNGKLPKHDPSFVQPGNRHYKYQCTWYAYNRRGQLGIPVPLWGDAADWIGGAKGAGYGVGRTPKQGACVIWQRGVQGGSPQYGHVAFVEKVLDGGKKIFISEHNYATPNGYGTRTIDMSSAIGKNAQFIYDKKSNSTSSSNNNGWKQNKDGIWYKAEHASFTVTAPEGIITRYKGPWTGHPQAGVLQKGQTIKYDEVQKFDGHVWVSWETFEGETVYMPVRTWDAKTGKVGKLWGEIK

SEQ ID NO: 79 - protein, 392 aa, Artificial Sequence
  M23LST_TCHAPK_SH3bAle1
AATHEHSAQWLNNYKKGYGYGPYPLGINGGMHYGVDFFMNIGTPVKAISSGKIVEAGWSNYGGGNQIGLIENDGVHRQWYMHLSKYNVKVGDYVKAGQIIGWSGSTGYSTAPHLHFQRMVNSFSNSTAQDPMPFLKSAGYGSNSTSSSNNNGSLKKYNGKLPKHDPSFVQPGNRHYKYQCTWYAYNRRGQLGIPVPLWGDAADWIGGAKGAGYGVGRTPKQGACVIWQRGVQGGSPQYGHVAFVEKVLDGGKKIFISEHNYATPNGYGTRTIDMSSAIGKNAQFIYDKKSNSTSSSNNNGYKTNKYGTLYKSESASFTANTDIITRLTGPFRSMPQSGVLRKGLTIKYDEVMKQDGHVWVGYNTNSGKRVYLPVRTWNESTGELGPLWGTIK

SEQ ID NO: 80 - protein, 392 aa, Artificial Sequence
  M23LST_TCHAPK_SH3bLST
AATHEHSAQWLNNYKKGYGYGPYPLGINGGMHYGVDFFMNIGTPVKAISSGKIVEAGWSNYGGGNQIGLIENDGVHRQWYMHLSKYNVKVGDYVKAGQIIGWSGSTGYSTAPHLHFQRMVNSFSNSTAQDPMPFLKSAGYGSNSTSSSNNNGSLKKYNGKLPKHDPSFVQPGNRHYKYQCTWYAYNRRGQLGIPVPLWGDAADWIGGAKGAGYGVGRTPKQGACVIWQRGVQGGSPQYGHVAFVEKVLDGGKKIFISEHNYATPNGYGTRTIDMSSAIGKNAQFIYDKKSNSTSSSNNNGWKTNKYGTLYKSESASFTPNTDIITRTTGPFRSMPQSGVLKAGQTIHYDEVMKQDGHVWVGYTGNSGQRIYLPVRTWNKSTNTLGVLWGTIK

SEQ ID NO: 81 - protein, 392 aa, Artificial Sequence
  M23LST_TCHAPTw_SH3b2638
AATHEHSAQWLNNYKKGYGYGPYPLGINGGMHYGVDFFMNIGTPVKAISSGKIVEAGWSNYGGGNQIGLIENDGVHRQWYMHLSKYNVKVGDYVKAGQIIGWSGSTGYSTAPHLHFQRMVNSFSNSTAQDPMPFLKSAGYGSNSTSSSNNNGGKELPTPRNKTDTSWTAPGNPNTGQWARECTWYCYNRRYELGLKAVAYGDAADWIAGARGAGISTGKEPKRGAVAVWARGVPGGSAQYGHVAFVEKVTDDGIYVSDYNYASPKTYGERLYKKGSPEYRNAQYIYDSNSTSSSNNNGWKQNKDGIWYKAEHASFTVTAPEGIITRYKGPWTGHPQAGVLQKGQTIKYDEVQKFDGHVWVSWETFEGETVYMPVRTWDAKTGKVGKLWGEIK

SEQ ID NO: 82 - protein, 390 aa, Artificial Sequence
  M23LST_TCHAPTw_SH3bAle1
AATHEHSAQWLNNYKKGYGYGPYPLGINGGMHYGVDFFMNIGTPVKAISSGKIVEAGWSNYGGGNQIGLIENDGVHRQWYMHLSKYNVKVGDYVKAGQIIGWSGSTGYSTAPHLHFQRMVNSFSNSTAQDPMPFLKSAGYGSNSTSSSNNNGGKELPTPRNKTDTSWTAPGNPNTGQWARECTWYCYNRRYELGLKAVAYGDAADWIAGARGAGISTGKEPKRGAVAVWARGVPGGSAQYGHVAFVEKVTDDGIYVSDYNYASPKTYGERLYKKGSPEYRNAQYIYDSNSTSSSNNNGYKTNKYGTLYKSESASFTANTDIITRLTGPFRSMPQSGVLRKGLTIKYDEVMKQDGHVWVGYNTNSGKRVYLPVRTWNESTGELGPLWGTIK

SEQ ID NO: 83 - protein, 390 aa, Artificial Sequence
  M23LST_TCHAPTw_SH3bLST
AATHEHSAQWLNNYKKGYGYGPYPLGINGGMHYGVDFFMNIGTPVKAISSGKIVEAGWSNYGGGNQIGLIENDGVHRQWYMHLSKYNVKVGDYVKAGQIIGWSGSTGYSTAPHLHFQRMVNSFSNSTAQDPMPFLKSAGYGSNSTSSSNNNGGKELPTPRNKTDTSWTAPGNPNTGQWARECTWYCYNRRYELGLKAVAYGDAADWIAGARGAGISTGKEPKRGAVAVWARGVPGGSAQYGHVAFVEKVTDDGIYVSDYNYASPKTYGERLYKKGSPEYRNAQYIYDSNSTSSSNNNGWKTNKYGTLYKSESASFTPNTDIITRTTGPFRSMPQSGVLKAGQTIHYDEVMKQDGHVWVGYTGNSGQRIYLPVRTWNKSTNTLGVLWGTIK